European Patent Application EP 4 252 743 A1, published October 4, 2023. Title: Exosomes expressing respiratory syncytial virus F protein and uses thereof. Applicant: KOREA INSTITUTE OF SCIENCE AND TECHNOLOGY. The sequence listing filed with the application follows.

SEQUENCE LISTING (2 sequences)

SEQ ID NO: 1 - protein, 574 aa, Unknown
  RSVF ORF
MELLIHRLSAIFLTLAINALYLTSSQNITEEFYQSTCSAVSRGYFSALRTGWYTSVITIELSNIKETKCNGTDTKVKLIKQELDKYKNAVTELQLLMQNTPAANNRARREAPQYMNYTINTTKNLNVSISKKRKRRFLGFLLGVGSAIASGIAVSKVLHLEGEVNKIKNALLSTNKAVVSLSNGVSVLTSKVLDLKNYINNQLLPIVNQQSCRISNIETVIEFQQKNSRLLEINREFSVNAGVTTPLSTYMLTNSELLSLINDMPITNDQKKLMSSNVQIVRQQSYSIMSIIKEEVLAYVVQLPIYGVIDTPCWKLHTSPLCTTNIKEGSNICLTRTDRGWYCDNAGSVSFFPQADTCKVQSNRVFCDTMNSLTLPSEVSLCNTDIFNSKYDCKIMTSKTDISSSVITSLGAIVSCYGKTKCTASNKNRGIIKTFSNGCDYVSNKGVDTVSVGNTLYYVNKLEGKNLYVKGEPIINYYDPLVFPSDEFDASISQVNEKINQSLAFIRRSDELLHNVNTGKSTTNIMITTIIIVIIVVLLSLIAIGLLLYCKAKNTPVTLSKDQLSGINNIAFSK

SEQ ID NO: 2 - DNA, 1722 bp, Unknown
  RSVF ORF
atggagctgcttattcacaggcttagcgctatttttttgaccttggccattaacgccttgtatctgacatcctcacagaatattacagaagaattttaccagtcaacctgctccgcggttagtagagggtatttctctgctctccggactggctggtatacatcagtcatcacgattgagttgtctaatatcaaggagacaaaatgcaatggcacagacaccaaagtgaaactcatcaagcaggagttggacaagtacaaaaatgctgtgacggaacttcaactgcttatgcagaatacacccgcggcaaacaatcgagcaaggagggaggctcctcagtacatgaattatacaattaatacaaccaagaaccttaatgtttcaatctcaaaaaaaagaaaaaggagatttctcgggttcctgttgggcgtgggctcagccattgcgagcgggattgctgtgtccaaggttctccacctggagggagaagtgaataagattaagaacgcgctcctgagtactaacaaggccgtcgtttctctcagcaatggggtgtcagtgctgacgagtaaagttctggacctgaaaaactatatcaacaatcagctgctgcccatcgtcaaccagcagagctgccgcattagcaacattgagaccgtaatcgagttccaacagaagaacagccggctcctggagatcaatcgagagttctccgttaatgctggtgttactacgccccttagcacttacatgttgacaaatagcgagctcctctccctgataaacgacatgccgattactaacgatcagaaaaagctgatgtctagtaacgtccagatcgtcagacagcagtcttattcaataatgagcataattaaggaagaagtattggcctacgtggtccaactgccaatctacggcgtgatcgataccccgtgctggaaacttcacactagccctctgtgtacgacaaatatcaaagagggatccaacatctgtcttacacgaaccgaccggggctggtattgcgacaacgccggtagcgtctcttttttcccacaggccgatacctgtaaggtgcagagcaatagggttttttgcgatacaatgaattccctgacgctgccctccgaagtaagcctgtgcaatacggatatcttcaattccaaatatgactgtaaaataatgacatcaaaaacagacatttcctccagcgtgatcaccagcctcggcgcaattgttagttgttacggcaaaacgaaatgcacggcctccaataagaatagagggatcattaaaaccttctcaaacggctgtgattacgtaagcaataagggcgtggacaccgtgagcgttggaaatactctctactacgtcaataaactggagggtaaaaacctctatgtcaagggcgagcctatcatcaattactatgatccattggtgtttcctagtgacgagttcgatgcatccatttcacaggttaacgagaagattaatcagtccctggcatttatccggcggagcgacgagctgctgcacaatgttaataccggtaagtccactactaacatcatgataaccacaattatcattgttatcatcgtcgtcttgctgagtcttattgctatcggccttctcctttattgcaaggccaagaatacaccggtgactctctctaaggaccaactgagtggaatcaataacattgcattctctaag